European Patent Specification EP 3 615 046 B1, published June 24, 2026. Title: CELLS EXPRESSING CHIMERIC ACTIVATING RECEPTORS AND CHIMERIC STIMULATING RECEPTORS AND USES THEREOF. Applicant: Eureka Therapeutics, Inc. Liu, Hong Zhang, Pengbo Horan, Lucas Xu, Yiyang Staley, Binnaz K. Liu, Lianxing Yun, Hongruo. Application Not Yet Assigned. The sequence listing filed with the application follows.

SEQUENCE LISTING (105 sequences)

SEQ ID NO: 1 - protein, 142 aa, Artificial Sequence
  Synthetic Construct
PNIQNPDPAVYQLRDSKSSDKSVCLFTDFDSQTNVSQSKDSDVYITDKTVLDMRSMDFKSNSAVAWSNKSDFACANAFNNSIIPEDTFFPSPESSCDVKLVEKSFETDTNLNFQNLSVIGFRILLLKVAGFNLLMTLRLWSS

SEQ ID NO: 2 - protein, 177 aa, Artificial Sequence
  Synthetic Construct
EDLNKVFPPEVAVFEPSEAEISHTQKATLVCLATGFFPDHVELSWWVNGKEVHSGVSTDPQPLKEQPALNDSRYCLSSRLRVSATFWQNPRNHFRCQVQFYGLSENDEWTQDRAKPVTQIVSAEAWGRADCGFTSVSYQQGVLSATILYEILLGKATLYAVLVSALVLMAMVKRKDF

SEQ ID NO: 3 - protein, 153 aa, Artificial Sequence
  Synthetic Construct
SQPHTKPSVFVMKNGTNVACLVKEFYPKDIRINLVSSKKITEFDPAIVISPSGKYNAVKLGKYEDSNSVTCSVQHDNKTVHSTDFEVKTDSTDHVKPKETENTKQPSKSCHKPKAIVHTEKVNMMSLTVLGLRMLFAKTVAVNFLLTAKLFFL

SEQ ID NO: 4 - protein, 173 aa, Artificial Sequence
  Synthetic Construct
DKQLDADVSPKPTIFLPSIAETKLQKAGTYLCLLEKFFPDVIKIHWQEKKSNTILGSQEGNTMKTNDTYMKFSWLTVPEKSLDKEHRCIVRHENNKNGVDQEIIFPPIKTDVITMDPKDNCSKDANDTLLLQLTNTSAYYMYLLLLLKSVVYFAIITCCLLRRTAFCCNGEKS

SEQ ID NO: 5 - protein, 20 aa, Artificial Sequence
  Synthetic Construct
ILLLKVAGFNLLMTLRLWSS

SEQ ID NO: 6 - protein, 23 aa, Artificial Sequence
  Synthetic Construct
TILYEILLGKATLYAVLVSALVL

SEQ ID NO: 7 - protein, 25 aa, Artificial Sequence
  Synthetic Construct
VLGLRMLFAKTVAVNFLLTAKLFFL

SEQ ID NO: 8 - protein, 23 aa, Artificial Sequence
  Synthetic Construct
YYMYLLLLLKSVVYFAIITCCLL

SEQ ID NO: 9 - protein, 25 aa, Artificial Sequence
  Synthetic Construct
VLGLRMLFAKTVAVNFLLTAKLFSL

SEQ ID NO: 10 - protein, 25 aa, Artificial Sequence
  Synthetic Construct
VLGLRVLFAKTVAVNFLLTAKLFFL

SEQ ID NO: 11 - protein, 25 aa, Artificial Sequence
  Synthetic Construct
VLGCRMLFAKTVAVNFLLTAKLFFL

SEQ ID NO: 12 - protein, 25 aa, Artificial Sequence
  Synthetic Construct
VLGLRMLFAKTFAVSFLLTAKLFFL

SEQ ID NO: 13 - protein, 25 aa, Artificial Sequence
  Synthetic Construct
VLGLRMLFAKTVAVNFLLTAKLFFS

SEQ ID NO: 14 - protein, 28 aa, Artificial Sequence
  Synthetic Construct
YYMYLLLLLKSVYYFAIITCCLLRRTAF

SEQ ID NO: 15 - protein, 28 aa, Artificial Sequence
  Synthetic Construct
YYMYLLLLLKSVVYFAIITCGLLRRTAF

SEQ ID NO: 16 - protein, 28 aa, Artificial Sequence
  Synthetic Construct
YLVYLLLLLKSVVYFVIVTCCLLRRTAF

SEQ ID NO: 17 - protein, 28 aa, Artificial Sequence
  Synthetic Construct
YLMYLLLLLKSVVYFAIITCCLLRRTAF

SEQ ID NO: 18 - protein, 28 aa, Artificial Sequence
  Synthetic Construct
YYVYLLLLLKSVVYFAIITCCLLRRTAF

SEQ ID NO: 19 - protein, 28 aa, Artificial Sequence
  Synthetic Construct
YYMYLLLLLKSVVYFVIITCCLLRRTAF

SEQ ID NO: 20 - protein, 28 aa, Artificial Sequence
  Synthetic Construct
YYMYLLLLLKSVVYFAIVTCCLLRRTAF

SEQ ID NO: 21 - protein, 28 aa, Artificial Sequence
  Synthetic Construct
YYIYLLLLLKSVVYFAIITCCLLRRTAF

SEQ ID NO: 22 - protein, 28 aa, Artificial Sequence
  Synthetic Construct
YIIYLLLLLKSVVYFIILTCCLLRRTAF

SEQ ID NO: 23 - protein, 28 aa, Artificial Sequence
  Synthetic Construct
YYMYCLLLLKSVVYFAIITCCLLRRTAF

SEQ ID NO: 24 - protein, 28 aa, Artificial Sequence
  Synthetic Construct
YYMYLLLFLKSFVYSAIITCCLLRRTAF

SEQ ID NO: 25 - protein, 28 aa, Artificial Sequence
  Synthetic Construct
YYMYLLLLLKSVVYFAIITMCLLRRTAF

SEQ ID NO: 26 - protein, 28 aa, Artificial Sequence
  Synthetic Construct
QYMYLLLLLKSVVYFAIITCCLLRRTAF

SEQ ID NO: 27 - protein, 30 aa, Artificial Sequence
  Synthetic Construct
ESSCDVKLVEKSFETDTNLNFQNLSVIGFR

SEQ ID NO: 28 - protein, 40 aa, Artificial Sequence
  Synthetic Construct
IPEDTFFPSPESSCDVKLVEKSFETDTNLNFQNLSVIGFR

SEQ ID NO: 29 - protein, 17 aa, Artificial Sequence
  Synthetic Construct
ADCGFTSVSYQQGVLSA

SEQ ID NO: 30 - protein, 19 aa, Artificial Sequence
  Synthetic Construct
GRADCGFTSVSYQQGVLSA

SEQ ID NO: 31 - protein, 41 aa, Artificial Sequence
  Synthetic Construct
DHVKPKETENTKQPSKSCHKPKAIVHTEKVNMMSLTVLGLR

SEQ ID NO: 32 - protein, 48 aa, Artificial Sequence
  Synthetic Construct
EVKTDSTDHVKPKETENTKQPSKSCHKPKAIVHTEKVNMMSLTVLGLR

SEQ ID NO: 33 - protein, 24 aa, Artificial Sequence
  Synthetic Construct
MDPKDNCSKDANDTLLLQLTNTSA

SEQ ID NO: 34 - protein, 32 aa, Artificial Sequence
  Synthetic Construct
PIKTDVITMDPKDNCSKDANDTLLLQLTNTSA

SEQ ID NO: 35 - protein, 9 aa, Artificial Sequence
  Synthetic Construct
MAMVKRKDF

SEQ ID NO: 36 - protein, 12 aa, Artificial Sequence
  Synthetic Construct
RRTAFCCNGEKS

SEQ ID NO: 37 - protein, 101 aa, Artificial Sequence
  Synthetic Construct
ASTKGPSVFPLAPSSKSTSGGTAALGCLVKDYFPEPVTVSWNSGALTSGVHTFPAVLQSSGSLSSVVTVPSSSLGTQTYICNVNHKPSNTKVDKRVEPKSC

SEQ ID NO: 38 - protein, 99 aa, Artificial Sequence
  Synthetic Construct
ASTKGPSVFPLAPCSRSTSESTAALGCLVKDYFPEPVTVSWNSGALTSGVHTFPAVLQSSGSLSSVVTVPSSNFGTQTYTCNVDHKPSNTKVDKTVERK

SEQ ID NO: 39 - protein, 100 aa, Artificial Sequence
  Synthetic Construct
ASTKGPSVFPLAPCSRSTSESTAALGCLVKDYFPEPVTVSWNSGALTSGVHTFPAVLQSSGSLSSVVTVPSSNFGTQTYTCNVDHKPSNTKVDKTVERKC

SEQ ID NO: 40 - protein, 101 aa, Artificial Sequence
  Synthetic Construct
ASTKGPSVFPLAPCSRSTSESTAALGCLVKDYFPEPVTVSWNSGALTSGVHTFPAVLQSSGSLSSVVTVPSSNFGTQTYTCNVDHKPSNTKVDKTVERKCC

SEQ ID NO: 41 - protein, 101 aa, Artificial Sequence
  Synthetic Construct
ASTKGPSVFPLAPCSRSTSGGTAALGCLVKDYFPEPVTVSWNSGALTSGVHTFPAVLQSSGSLSSVVTVPSSSLGTQTYTCNVNHKPSNTKVDKRVELKTP

SEQ ID NO: 42 - protein, 101 aa, Artificial Sequence
  Synthetic Construct
ASTKGPSVFPLAPCSRSTSESTAALGCLVKDYFPEPVTVSWNSGALTSGVHTFPAVLQSSGSLSSVVTVPSSSLGTKTYTCNVDHKPSNTKVDKRVESKYG

SEQ ID NO: 43 - protein, 119 aa, Artificial Sequence
  Synthetic Construct
DTSPKVFPLSLCSTQPDGNVVIACLVQGFFPQEPLSVTWSESGQGVTARNFPPSQDASGDLYTTSSQLTLPATQCLAGKSVTCHVKHYTNPSQDVTVPCPVPSTPPTPSPSTPPTPSPS

SEQ ID NO: 44 - protein, 106 aa, Artificial Sequence
  Synthetic Construct
DTSPKVFPLSLDSTPQDGNVVVACLVQGFFPQEPLSVTWSESGQNVTARNFPPSQDASGDLYTTSSQLTLPATQCPDGKSVTCHVKHYTNPSQDVTVPCPVPPPPP

SEQ ID NO: 45 - protein, 159 aa, Artificial Sequence
  Synthetic Construct
APTKAPDVFPIISGCRHPKDNSPVVLACLITGYHPTSVTVTWYMGTQSQPQRTFPEIQRRDSYYMTSSQLSTPLQQWRQGEYKCVVQHTASKSKKEIFRWPESPKAQASSVPTAQPQAEGSLAKATTAPATTRNTGRGGEEKKKEKEKEEQEERETKTP

SEQ ID NO: 46 - protein, 103 aa, Artificial Sequence
  Synthetic Construct
ASTQSPSVFPLTRCCKNIPSNATSVTLGCLATGYFPEPVMVTWDTGSLNGTTMTLPATTLTLSGHYATISLLTVSGAWAKQMFTCRVAHTPSSTDWVDNKTFS

SEQ ID NO: 47 - protein, 104 aa, Artificial Sequence
  Synthetic Construct
GSASAPTLFPLVSCENSPSDTSSVAVGCLAQDFLPDSITLSWKYKNNSDISSTRGFPSVLRGGKYAATSQVLLPSKDVMQGTDEHVVCKVQHPNGNKEKNVPLP

SEQ ID NO: 48 - protein, 106 aa, Artificial Sequence
  Synthetic Construct
GQPKANPTVTLFPPSSEELQANKATLVCLISDFYPGAVTVAWKADGSPVKAGVETTKPSKQSNNKYAASSYLSLTPEQWKSHRSYSCQVTHEGSTVEKTVAPTECS

SEQ ID NO: 49 - protein, 105 aa, Artificial Sequence
  Synthetic Construct
IEVMYPPPYLDNEKSNGTIIHVKGKHLCPSPLFPGPSKPFWVLVVVGGVLACLLVTVAFIIFWVRSKRSRLLHSDYMNMTPRRPGPTRKHYQPYAPPRDFAAYRS

SEQ ID NO: 50 - protein, 108 aa, Artificial Sequence
  Synthetic Construct
RVKFSRSADAPAYQQGQNQLYNELNLGRREEYDVLDKRRGRDPEMGGKPRRKNPQEGNELQKDKMAEAYSEIGMKGERRRGKGHDGQGLSTATKDTYDALHMQALPPR

SEQ ID NO: 51 - protein, 105 aa, Artificial Sequence; identical to SEQ ID NO: 49
  Synthetic Construct

SEQ ID NO: 52 - protein, 41 aa, Artificial Sequence
  Synthetic Construct
RSKRSRLLHSDYMNMTPRRPGPTRKHYQPYAPPRDFAAYRS

SEQ ID NO: 53 - protein, 94 aa, Artificial Sequence
  Synthetic Construct
PADLSPGASSVTPPAPAREPGHSPQIISFFLALTSTALLFLLFFLTLRFSVVKRGRKKLLYIFKQPFMRPVQTTQEEDGCSCRFPEEEEGGCEL

SEQ ID NO: 54 - protein, 42 aa, Artificial Sequence
  Synthetic Construct
KRGRKKLLYIFKQPFMRPVQTTQEEDGCSCRFPEEEEGGCEL

SEQ ID NO: 55 - protein, 106 aa, Artificial Sequence
  Synthetic Construct
DPPATQPQETQGPPARPITVQPTEAWPRTSQGPSWVEVPGGRAVAAILGLGLVLGLLGPLAILLALYLLRRDQRLPPDAHKPPGGGSFRTPIQEEQADAHSTLAKI

SEQ ID NO: 56 - protein, 42 aa, Artificial Sequence
  Synthetic Construct
ALYLLRRDQRLPPDAHKPPGGGSFRTPIQEEQADAHSTLAKI

SEQ ID NO: 57 - protein, 69 aa, Artificial Sequence
  Synthetic Construct
TTTPAPRPPTPAPTIASQPLSLRPEACRPAAGGAVHTRGLDFACDIYIWAPLAGTCGVLLLSLVITLYC

SEQ ID NO: 58 - protein, 130 aa, Artificial Sequence
  Synthetic Construct
EVQLVQSGAEVKKPGESLKISCKGSGYSFTSYWIGWVRQMPGKGLEWMGIIYPGDSDTRYSPSFQGQVTISADKSISTAYLQWSSLKASDTAMYYCARQVWGWQGGMYPRSNWWYNLDSWGQGTLVTVSS

SEQ ID NO: 59 - protein, 109 aa, Artificial Sequence
  Synthetic Construct
LPVLTQPPSVSVAPGKTARITCGGNNIGSKSVHWYQQKPGQAPVLVVYDDSDRPSGIPERFSGSNSGNTATLTISRVEAGDEADYYCQVWDSSSDYVVFGGGTKLTVLG

SEQ ID NO: 60 - protein, 121 aa, Artificial Sequence
  Synthetic Construct
QVQLQQPGAELVKPGASVKMSCKASGYTFTSYNMHWVKQTPGRGLEWIGAIYPGNGDTSYNQKFKGKATLTADKSSSTAYMQLSSLTSEDSAVYYCARSTYYGGDWYFNVWGAGTTVTVSS

SEQ ID NO: 61 - protein, 105 aa, Artificial Sequence
  Synthetic Construct
QIVLSQSPAILSDGEKVTMTCRASSSVSYIHWFQQKPGSSPKPWIYATSNLASGVPVRFSGSGSGTSYSLTISRVEAEDAATYYCQQWTSNPPTFGGGTKLEIKR

SEQ ID NO: 62 - protein, 117 aa, Artificial Sequence
  Synthetic Construct
EVQLVQSGAEVKKPGESLTISCKASGYSFPNYWITWVRQMSGGGLEWMGRIDPGDSYTTYNPSFQGHVTISIDKSTNTAYLHWNSLKASDTAMYYCARYYVSLVDIWGQGTLVTVSS

SEQ ID NO: 63 - protein, 110 aa, Artificial Sequence
  Synthetic Construct
QSVLTQPASVSGSPGQSITISCTGTSSDVGGYNYVSWYQQHPGKAPKLMIYDVNNRPSEVSNRFSGSKSGNTASLTISGLQAEDEADYYCSSYTTGSRAVFGGGTKLTVL

SEQ ID NO: 64 - protein, 118 aa, Artificial Sequence
  Synthetic Construct
QVQLVESGGGLVQPGGSLRLSCAASGFTFSSYAMSWVRQAPGKGLEWVSVIYSGGSSTYYADSVKGRFTISRDNSKNTLYLQMNSLRAEDTAVYYCARTSYLNHGDYWGQGTLVTVSS

SEQ ID NO: 65 - protein, 111 aa, Artificial Sequence
  Synthetic Construct
QSVLTQPPSVSAAPGQRVTISCSGTRSNIGSDYVSWYQHLPGTAPKLLVYGDNLRPSGIPDRFSASKSGTSATLGITGLQTGDEADYYCGTWDYTLNGVVFGGGTKLTVLG

SEQ ID NO: 66 - protein, 112 aa, Artificial Sequence
  Synthetic Construct
QVQLQESGPGLVKPSQTLSLTCTVSGYTFTNYYVFWVRQRQRLEWIGDINPVNGDTNFNEKFKNRVTISADKSISTAYLQWSSLKASDTAMYYCRGYTMDYWGQGTLVTVSS

SEQ ID NO: 67 - protein, 113 aa, Artificial Sequence
  Synthetic Construct
DIVMTQTPLSLPVTPGEPASISCRSSQSLVHSNGNTYLHWYQQKPGKAPKLLIYKVSYRFSGVPDRFSGSGSGTDFTLKISRVEAEDVGVYYCSQNTHVPRTFGQGTKVEIKR

SEQ ID NO: 68 - protein, 286 aa, Artificial Sequence
  Synthetic Construct
EVQLVQSGAEVKKPGESLTISCKASGYSFPNYWITWVRQMSGGGLEWMGRIDPGDSYTTYNPSFQGHVTISIDKSTNTAYLHWNSLKASDTAMYYCARYYVSLVDIWGQGTLVTVSSASTKGPSVFPLAPSSKSTSGGTAALGCLVKDYFPEPVTVSWNSGALTSGVHTFPAVLQSSGSLSSVVTVPSSSLGTQTYICNVNHKPSNTKVDKRVEPKSCEVKTDSTDHVKPKETENTKQPSKSCHKPKAIVHTEKVNMMSLTVLGLRMLFAKTVAVNFLLTAKLFFL

SEQ ID NO: 69 - protein, 283 aa, Artificial Sequence
  Synthetic Construct
QSVLTQPASVSGSPGQSITISCTGTSSDVGGYNYVSWYQQHPGKAPKLMIYDVNNRPSEVSNRFSGSKSGNTASLTISGLQAEDEADYYCSSYTTGSRAVFGGGTKLTVLGQPKANPTVTLFPPSSEELQANKATLVCLISDFYPGAVTVAWKADGSPVKAGVETTKPSKQSNNKYAASSYLSLTPEQWKSHRSYSCQVTHEGSTVEKTVAPTECSPIKTDVITMDPKDNCSKDANDTLLLQLTNTSAYYMYLLLLLKSVVYFAIITCCLLRRTAFCCNGEKS

SEQ ID NO: 70 - protein, 286 aa, Artificial Sequence
  Synthetic Construct
EVQLVQSGAEVKKPGESLTISCKASGYSFPNYWITWVRQMSGGGLEWMGRIDPGDSYTTYNPSFQGHVTISIDKSTNTAYLHWNSLKASDTAMYYCARYYVSLVDIWGQGTLVTVSSASTKGPSVFPLAPSSKSTSGGTAALGCLVKDYFPEPVTVSWNSGALTSGVHTFPAVLQSSGSLSSVVTVPSSSLGTQTYICNVNHKPSNTKVDKRVEPKSCEVKTDSTDHVKPKETENTKQPSKSCHKPKAIVHTEKVNMMSLTVLGLRVLFAKTVAVNFLLTAKLFFL

SEQ ID NO: 71 - protein, 283 aa, Artificial Sequence
  Synthetic Construct
QSVLTQPASVSGSPGQSITISCTGTSSDVGGYNYVSWYQQHPGKAPKLMIYDVNNRPSEVSNRFSGSKSGNTASLTISGLQAEDEADYYCSSYTTGSRAVFGGGTKLTVLGQPKANPTVTLFPPSSEELQANKATLVCLISDFYPGAVTVAWKADGSPVKAGVETTKPSKQSNNKYAASSYLSLTPEQWKSHRSYSCQVTHEGSTVEKTVAPTECSPIKTDVITMDPKDNCSKDANDTLLLQLTNTSAYLVYLLLLLKSVVYFVIVTCCLLRRTAFCCNGEKS

SEQ ID NO: 72 - protein, 299 aa, Artificial Sequence
  Synthetic Construct
EVQLVQSGAEVKKPGESLKISCKGSGYSFTSYWIGWVRQMPGKGLEWMGIIYPGDSDTRYSPSFQGQVTISADKSISTAYLQWSSLKASDTAMYYCARQVWGWQGGMYPRSNWWYNMDSWGQGTLVTVSSASTKGPSVFPLAPSSKSTSGGTAALGCLVKDYFPEPVTVSWNSGALTSGVHTFPAVLQSSGSLSSVVTVPSSSLGTQTYICNVNHKPSNTKVDKRVEPKSCEVKTDSTDHVKPKETENTKQPSKSCHKPKAIVHTEKVNMMSLTVLGLRMLFAKTVAVNFLLTAKLFFL

SEQ ID NO: 73 - protein, 281 aa, Artificial Sequence
  Synthetic Construct
LPVLTQPPSVSVAPGKTARITCGGNNIGSKSVHWYQQKPGQAPVLVVYDDSNRPSGIPERFSGSNSGNTATLTISRVEAGDEADYYCQVWDSSSEYVVFGGGTKLTVLGQPKANPTVTLFPPSSEELQANKATLVCLISDFYPGAVTVAWKADGSPVKAGVETTKPSKQSNNKYAASSYLSLTPEQWKSHRSYSCQVTHEGSTVEKTVAPTECSPIKTDVITMDPKDNCSKDANDTLLLQLTNTSAYYMYLLLLLKSVVYFAIITCCLLRRTAFCCNGEKS

SEQ ID NO: 74 - protein, 299 aa, Artificial Sequence
  Synthetic Construct
EVQLVQSGAEVKKPGESLKISCKGSGYSFTSYWIGWVRQMPGKGLEWMGIIYPGDSDTRYSPSFQGQVTISADKSISTAYLQWSSLKASDTAMYYCARQVWGWQGGMYPRSNWWYNMDSWGQGTLVTVSSASTKGPSVFPLAPSSKSTSGGTAALGCLVKDYFPEPVTVSWNSGALTSGVHTFPAVLQSSGSLSSVVTVPSSSLGTQTYICNVNHKPSNTKVDKRVEPKSCEVKTDSTDHVKPKETENTKQPSKSCHKPKAIVHTEKVNMMSLTVLGLRVLFAKTVAVNFLLTAKLFFL

SEQ ID NO: 75 - protein, 281 aa, Artificial Sequence
  Synthetic Construct
LPVLTQPPSVSVAPGKTARITCGGNNIGSKSVHWYQQKPGQAPVLVVYDDSNRPSGIPERFSGSNSGNTATLTISRVEAGDEADYYCQVWDSSSEYVVFGGGTKLTVLGQPKANPTVTLFPPSSEELQANKATLVCLISDFYPGAVTVAWKADGSPVKAGVETTKPSKQSNNKYAASSYLSLTPEQWKSHRSYSCQVTHEGSTVEKTVAPTECSPIKTDVITMDPKDNCSKDANDTLLLQLTNTSAYLVYLLLLLKSVVYFVIVTCCLLRRTAFCCNGEKS

SEQ ID NO: 76 - protein, 21 aa, Artificial Sequence
  Synthetic Construct
SRGGGGSGGGGSGGGGSLEMA

SEQ ID NO: 77 - protein, 260 aa, Artificial Sequence
  Synthetic Construct
LPVLTQPPSVSVAPGKTARITCGGNNIGSKSVHWYQQKPGQAPVLVVYDDSDRPSGIPERFSGSNSGNTATLTISRVEAGDEADYYCQVWDSSSDYVVFGGGTKLTVLGSRGGGGSGGGGSGGGGSLEMAEVQLVQSGAEVKKPGESLKISCKGSGYSFTSYWIGWVRQMPGKGLEWMGIIYPGDSDTRYSPSFQGQVTISADKSISTAYLQWSSLKASDTAMYYCARQVWGWQGGMYPRSNWWYNLDSWGQGTLVTVSS

SEQ ID NO: 78 - protein, 245 aa, Artificial Sequence
  Synthetic Construct
QIVLSQSPAILSDGEKVTMTCRASSSVSYIHWFQQKPGSSPKPWIYATSNLASGVPVRFSGSGSGTSYSLTISRVEAEDAATYYCQQWTSNPPTFGGGTKLEIKRSRGGGGSGGGGSGGGGSLEQVQLQQPGAELVKPGASVKMSCKASGYTFTSYNMHWVKQTPGRGLEWIGAIYPGNGDTSYNQKFKGKATLTADKSSSTAYMQLSSLTSEDSAVYYCARSTYYGGDWYFNVWGAGTTVTVSS

SEQ ID NO: 79 - protein, 250 aa, Artificial Sequence
  Synthetic Construct
QSVLTQPPSVSAAPGQRVTISCSGTRSNIGSDYVSWYQHLPGTAPKLLVYGDNLRPSGIPDRFSASKSGTSATLGITGLQTGDEADYYCGTWDYTLNGVVFGGGTKLTVLGSRGGGGSGGGGSGGGGSLEMAQVQLVESGGGLVQPGGSLRLSCAASGFTFSSYAMSWVRQAPGKGLEWVSVIYSGGSSTYYADSVKGRFTISRDNSKNTLYLQMNSLRAEDTAVYYCARTSYLNHGDYWGQGTLVTVSS

SEQ ID NO: 80 - protein, 368 aa, Artificial Sequence
  Synthetic Construct
LPVLTQPPSVSVAPGKTARITCGGNNIGSKSVHWYQQKPGQAPVLVVYDDSDRPSGIPERFSGSNSGNTATLTISRVEAGDEADYYCQVWDSSSDYVVFGGGTKLTVLGSRGGGGSGGGGSGGGGSLEMAEVQLVQSGAEVKKPGESLKISCKGSGYSFTSYWIGWVRQMPGKGLEWMGIIYPGDSDTRYSPSFQGQVTISADKSISTAYLQWSSLKASDTAMYYCARQVWGWQGGMYPRSNWWYNLDSWGQGTLVTVSSAAAIEVMYPPPYLDNEKSNGTIIHVKGKHLCPSPLFPGPSKPFWVLVVVGGVLACLLVTVAFIIFWVRSKRSRLLHSDYMNMTPRRPGPTRKHYQPYAPPRDFAAYRS

SEQ ID NO: 81 - protein, 353 aa, Artificial Sequence
  Synthetic Construct
QIVLSQSPAILSDGEKVTMTCRASSSVSYIHWFQQKPGSSPKPWIYATSNLASGVPVRFSGSGSGTSYSLTISRVEAEDAATYYCQQWTSNPPTFGGGTKLEIKRSRGGGGSGGGGSGGGGSLEQVQLQQPGAELVKPGASVKMSCKASGYTFTSYNMHWVKQTPGRGLEWIGAIYPGNGDTSYNQKFKGKATLTADKSSSTAYMQLSSLTSEDSAVYYCARSTYYGGDWYFNVWGAGTTVTVSSAAAIEVMYPPPYLDNEKSNGTIIHVKGKHLCPSPLFPGPSKPFWVLVVVGGVLACLLVTVAFIIFWVRSKRSRLLHSDYMNMTPRRPGPTRKHYQPYAPPRDFAAYRS

SEQ ID NO: 82 - protein, 358 aa, Artificial Sequence
  Synthetic Construct
QSVLTQPPSVSAAPGQRVTISCSGTRSNIGSDYVSWYQHLPGTAPKLLVYGDNLRPSGIPDRFSASKSGTSATLGITGLQTGDEADYYCGTWDYTLNGVVFGGGTKLTVLGSRGGGGSGGGGSGGGGSLEMAQVQLVESGGGLVQPGGSLRLSCAASGFTFSSYAMSWVRQAPGKGLEWVSVIYSGGSSTYYADSVKGRFTISRDNSKNTLYLQMNSLRAEDTAVYYCARTSYLNHGDYWGQGTLVTVSSAAAIEVMYPPPYLDNEKSNGTIIHVKGKHLCPSPLFPGPSKPFWVLVVVGGVLACLLVTVAFIIFWVRSKRSRLLHSDYMNMTPRRPGPTRKHYQPYAPPRDFAAYRS

SEQ ID NO: 83 - DNA, 180 bp, Artificial Sequence
  Synthetic Construct
ggaggaaaaactgtttcatacagaaggcgtggaggaaaaactgtttcatacagaaggcgtggaggaaaaactgtttcatacagaaggcgtggaggaaaaactgtttcatacagaaggcgtggaggaaaaactgtttcatacagaaggcgtggaggaaaaactgtttcatacagaaggcgt

SEQ ID NO: 84 - DNA, 149 bp, Artificial Sequence
  Synthetic Construct
gccgccccgactgcatctgcgtgttccaattcgccaatgacaagacgctgggcggggtttgtgtcatcatagaactaaagacatgcaaatatatttcttccggggacaccgccagcaaacgcgagcaacgggccacggggatgaagcag

SEQ ID NO: 85 - DNA, 335 bp, Artificial Sequence
  Synthetic Construct
ggaggaaaaactgtttcatacagaaggcgtggaggaaaaactgtttcatacagaaggcgtggaggaaaaactgtttcatacagaaggcgtggaggaaaaactgtttcatacagaaggcgtggaggaaaaactgtttcatacagaaggcgtggaggaaaaactgtttcatacagaaggcgtctcgaggccgccccgactgcatctgcgtgttccaattcgccaatgacaagacgctgggcggggtttgtgtcatcatagaactaaagacatgcaaatatatttcttccggggacaccgccagcaaacgcgagcaacgggccacggggatgaagcag

SEQ ID NO: 86 - protein, 119 aa, Artificial Sequence
  Synthetic Construct
PTHLPYVSEMLEARTAGHMQTLADFRQLPARTLSTHWPPQRSLCSSDFIRILVIFSGMFLVFTLAGALFLHQRRKYRSNKGESPVEPAEPCRYSCPREEEGSTIPIQEDYRKPEPACSP

SEQ ID NO: 87 - protein, 48 aa, Artificial Sequence
  Synthetic Construct
QRRKYRSNKGESPVEPAEPCRYSCPREEEGSTIPIQEDYRKPEPACSP

SEQ ID NO: 88 - protein, 264 aa, Artificial Sequence
  Synthetic Construct
APPLGTQPDCNPTPENGEAPASTSPTQSLLVDSQASKTLPIPTSAPVSSTGKPVLDAGPVLFWVILVLVVVVGSSAFLLCHRRACRKRIRQKLHLCYPVQTSQPKLELVDSRPRRSSTQLRSGASVTEPVAEERGLMSQPLMCHSVGAAYLESLPLQDDAGGPSSPRDLPEPRVSTEHTNNKIEKIYIMKADTVIVGTVKAELPEGRGLAGPAEPELEEELEADHTPHYPEQETEPPLGSCSDVMLSVEEEGKEDPLPTAASGK

SEQ ID NO: 89 - protein, 184 aa, Artificial Sequence
  Synthetic Construct
HRRACRKRIRQKLHLCYPVQTSQPKLELVDSRPRRSSTQLRSGASVTEPVAEERGLMSQPLMCHSVGAAYLESLPLQDDAGGPSSPRDLPEPRVSTEHTNNKIEKIYIMKADTVIVGTVKAELPEGRGLAGPAEPELEEELEADHTPHYPEQETEPPLGSCSDVMLSVEEEGKEDPLPTAASGK

SEQ ID NO: 90 - protein, 108 aa, Artificial Sequence
  Synthetic Construct
AAAIEVMYPPPYLDNEKSNGTIIHVKGKHLCPSPLFPGPSKPFWVLVVVGGVLACLLVTVAFIIFWVRSKRSRLLHSDYMNMTPRRPGPTRKHYQPYAPPRDFAAYRS

SEQ ID NO: 91 - protein, 116 aa, Artificial Sequence
  Synthetic Construct
AAATGTTTPAPRPPTPAPTIASQPLSLRPEACRPAAGGAVHTRGLDFACDIYIWAPLAGTCGVLLLSLVITLYCKRGRKKLLYIFKQPFMRPVQTTQEEDGCSCRFPEEEEGGCEL

SEQ ID NO: 92 - protein, 99 aa, Artificial Sequence
  Synthetic Construct
AAATGPADLSPGASSVTPPAPAREPGHSPQIISFFLALTSTALLFLLFFLTLRFSVVKRGRKKLLYIFKQPFMRPVQTTQEEDGCSCRFPEEEEGGCEL

SEQ ID NO: 93 - protein, 122 aa, Artificial Sequence
  Synthetic Construct
AAATGTTTPAPRPPTPAPTIASQPLSLRPEACRPAAGGAVHTRGLDFACDIYIWAPLAGTCGVLLLSLVITLYCQRRKYRSNKGESPVEPAEPCRYSCPREEEGSTIPIQEDYRKPEPACSP

SEQ ID NO: 94 - protein, 124 aa, Artificial Sequence
  Synthetic Construct
AAATGPTHLPYVSEMLEARTAGHMQTLADFRQLPARTLSTHWPPQRSLCSSDFIRILVIFSGMFLVFTLAGALFLHQRRKYRSNKGESPVEPAEPCRYSCPREEEGSTIPIQEDYRKPEPACSP

SEQ ID NO: 95 - protein, 258 aa, Artificial Sequence
  Synthetic Construct
AAATGTTTPAPRPPTPAPTIASQPLSLRPEACRPAAGGAVHTRGLDFACDIYIWAPLAGTCGVLLLSLVITLYCHRRACRKRIRQKLHLCYPVQTSQPKLELVDSRPRRSSTQLRSGASVTEPVAEERGLMSQPLMCHSVGAAYLESLPLQDDAGGPSSPRDLPEPRVSTEHTNNKIEKIYIMKADTVIVGTVKAELPEGRGLAGPAEPELEEELEADHTPHYPEQETEPPLGSCSDVMLSVEEEGKEDPLPTAASGK

SEQ ID NO: 96 - protein, 269 aa, Artificial Sequence
  Synthetic Construct
AAATGAPPLGTQPDCNPTPENGEAPASTSPTQSLLVDSQASKTLPIPTSAPVSSTGKPVLDAGPVLFWVILVLVVVVGSSAFLLCHRRACRKRIRQKLHLCYPVQTSQPKLELVDSRPRRSSTQLRSGASVTEPVAEERGLMSQPLMCHSVGAAYLESLPLQDDAGGPSSPRDLPEPRVSTEHTNNKIEKIYIMKADTVIVGTVKAELPEGRGLAGPAEPELEEELEADHTPHYPEQETEPPLGSCSDVMLSVEEEGKEDPLPTAASGK

SEQ ID NO: 97 - protein, 116 aa, Artificial Sequence
  Synthetic Construct
AAATGTTTPAPRPPTPAPTIASQPLSLRPEACRPAAGGAVHTRGLDFACDIYIWAPLAGTCGVLLLSLVITLYCALYLLRRDQRLPPDAHKPPGGGSFRTPIQEEQADAHSTLAKI

SEQ ID NO: 98 - protein, 113 aa, Artificial Sequence
  Synthetic Construct
AAATGDRDPPATQPQETQGPPARPITVQPTEAWPRTSQGPSWVEVPGGRAVAAILGLGLVLGLLGPLAILLALYLLRRDQRLPPDAHKPPGGGSFRTPIQEEQADAHSTLAKI

SEQ ID NO: 99 - protein, 129 aa, Artificial Sequence
  Synthetic Construct
EVQLVQSGAEVKKPGESLKISCKGSGYSFTSYWIGWVRQMPGKGLEWMGIIYPGDSDTRYSPSFQGQVTIADKSISTAYLQWSSLKASDTAMYYCARQVWGWQGGMYPRSNWWYNLDSWGQGTLVTVSS

SEQ ID NO: 100 - protein, 108 aa, Artificial Sequence
  Synthetic Construct
LPVLTQPPSVSVAPGKTARITCGGNNIGSKSVHWYQQKPGQAPVLVVYDDSDRPSGIPERFSGSNSGNTATLTISRVEAGDEADYYCQVWDSSSDYVVFGGGTKLTVL

SEQ ID NO: 101 - protein, 118 aa, Artificial Sequence
  Synthetic Construct
QVQLVESGGGLVQPGGSLRLSCAASGFTFSNYAMSWVRQAPGKGLEWVSSISGSGGSTYYADSVKGRFTISRDTSKNTLYLQMNSLRAEDTAVYYCARYGSAAWMDSWGQGTLVTVSS

SEQ ID NO: 102 - protein, 106 aa, Artificial Sequence
  Synthetic Construct
DIQLTQSPSSLSTSVGDRVTITCQASHDIRNYLNWYQQKPGKAPNLLIYANLQTGVPSRFSGRGSGTDFTLTISSLQPEDIATYYCQQYDGLPLTFGQGTRLEIKR

SEQ ID NO: 103 - protein, 3 aa, Artificial Sequence
  Synthetic Construct
AAA

SEQ ID NO: 104 - protein, 5 aa, Artificial Sequence
  Synthetic Construct
AAATG

SEQ ID NO: 105 - protein, 500 aa, Artificial Sequence
  Synthetic Construct
QSVLTQPPSVSAAPGQRVTISCSGTRSNIGSDYVSWYQHLPGTAPKLLVYGDNLRPSGIPDRFSASKSGTSATLGITGLQTGDEADYYCGTWDYTLNGVVFGGGTKLTVLGSRGGGGSGGGGSGGGGSLEMAQVQLVESGGGLVQPGGSLRLSCAASGFTFSSYAMSWVRQAPGKGLEWVSVIYSGGSSTYYADSVKGRFTISRDNSKNTLYLQMNSLRAEDTAVYYCARTSYLNHGDYWGQGTLVTVSSTSGGGGSDVQLVQSGAEVKKPGASVKVSCKASGYTFTRYTMHWVRQAPGQGLEWIGYINPSRGYTNYADSVKGRFTITTDKSTSTAYMELSSLRSEDTATYYCARYYDDHYCLDYWGQGTTVTVSSGEGTSTGSGGSGGSGGADDIVLTQSPATLSLSPGERATLSCRASQSVSYMNWYQQKPGKAPKRWIYDTSKVASGVPARFSGSGSGTDYSLTINSLEAEDAATYYCQQWSSNPLTFGGGTKVEIK